European Patent Specification EP 3 478 723 B1, published December 17, 2025. Title: PD-L1-SPECIFIC ANTIBODIES AND METHODS OF USING THE SAME. Applicant: CHECKPOINT THERAPEUTICS, INC. The sequence listing filed with the application follows.

SEQUENCE LISTING (78 sequences)

SEQ ID NO: 1 - protein, 9 aa, Homo sapiens
GTFSSYAIS

SEQ ID NO: 2 - protein, 9 aa, Homo sapiens
GTFSRSAIS

SEQ ID NO: 3 - protein, 9 aa, Homo sapiens
GTFSGYAIS

SEQ ID NO: 4 - protein, 9 aa, Homo sapiens
GTFWRYAIS

SEQ ID NO: 5 - protein, 9 aa, Homo sapiens
GTFGSYAIS

SEQ ID NO: 6 - protein, 9 aa, Homo sapiens
GTFGTYAIS

SEQ ID NO: 7 - protein, 9 aa, Homo sapiens
GTFSPKAIS

SEQ ID NO: 8 - protein, 17 aa, Homo sapiens
GIIPIFGTANYAQKFQG

SEQ ID NO: 9 - protein, 17 aa, Homo sapiens
VIIPAFGEANYAQKFQG

SEQ ID NO: 10 - protein, 17 aa, Homo sapiens
VIIPAFGTANYAQKFQG

SEQ ID NO: 11 - protein, 17 aa, Homo sapiens
VIIPIWGKANYAQKFQG

SEQ ID NO: 12 - protein, 17 aa, Homo sapiens
GIYPAFGTANYAQKFQG

SEQ ID NO: 13 - protein, 17 aa, Homo sapiens
GIYPRFGTANYAQKFQG

SEQ ID NO: 14 - protein, 17 aa, Homo sapiens
VIIPIFGPANYAQKFQG

SEQ ID NO: 15 - protein, 13 aa, Homo sapiens
ARGRQMFGAGIDF

SEQ ID NO: 16 - protein, 9 aa, Homo sapiens
YTLSSHGIT

SEQ ID NO: 17 - protein, 17 aa, Homo sapiens
WISAHSGHASNAQKVED

SEQ ID NO: 18 - protein, 13 aa, Homo sapiens
ARVWRALYHGMDV

SEQ ID NO: 19 - protein, 13 aa, Homo sapiens
ARVHAALYHGMDV

SEQ ID NO: 20 - protein, 13 aa, Homo sapiens
TRSSGSIDSNYVQ

SEQ ID NO: 21 - protein, 7 aa, Homo sapiens
EDNQRPS

SEQ ID NO: 22 - protein, 11 aa, Homo sapiens
QSYDSNNRHVI

SEQ ID NO: 23 - protein, 11 aa, Homo sapiens
GGNNIGSKGVH

SEQ ID NO: 24 - protein, 7 aa, Homo sapiens
DDSDRPS

SEQ ID NO: 25 - protein, 11 aa, Homo sapiens
QVWDSSSDHWV

SEQ ID NO: 26 - protein, 26 aa, Homo sapiens
EVQLVQSGAEVKKPGSSVKVSCKASG

SEQ ID NO: 27 - protein, 26 aa, Homo sapiens
QVQLVQSGAEVKKPGSSVKVSCKASG

SEQ ID NO: 28 - protein, 14 aa, Homo sapiens
WVRQAPGQGLEWMG

SEQ ID NO: 29 - protein, 30 aa, Homo sapiens
RVTITADKSTSTAYMELSSLRSEDTAVYYC

SEQ ID NO: 30 - protein, 11 aa, Homo sapiens
WGQGTLVTVSS

SEQ ID NO: 31 - protein, 22 aa, Homo sapiens
NFMLTQPHSVSESPGKTVTISC

SEQ ID NO: 32 - protein, 15 aa, Homo sapiens
WYQQRPGSAPTTVIY

SEQ ID NO: 33 - protein, 34 aa, Homo sapiens
GVPDRFSGSIDSSSNSASLTISGLKTEDEADYYC

SEQ ID NO: 34 - protein, 10 aa, Homo sapiens
FGGGTKLTVL

SEQ ID NO: 35 - protein, 120 aa, Homo sapiens
EVQLVQSGAEVKKPGSSVKVSCKASGGTFSSYAISWVRQAPGQGLEWMGGIIPIFGTANYAQKFQGRVTITADKSTSTAYMELSSLRSEDTAVYYCARGRQMFGAGIDFWGQGTLVTVSS

SEQ ID NO: 36 - protein, 120 aa, Homo sapiens
QVQLVQSGAEVKKPGSSVKVSCKASGGTFSRSAISWVRQAPGQGLEWMGVIIPAFGEANYAQKFQGRVTITADESTSTAYMELSSLRSEDTAVYYCARGRQMFGAGIDFWGQGTLVTVSS

SEQ ID NO: 37 - protein, 120 aa, Homo sapiens
QVQLVQSGAEVKKPGSSVKVSCKASGGTFSGYAISWVRQAPGQGLEWMGVIIPAFGTANYAQKFQGRVTITADESTSTAYMELSSLRSEDTAVYYCARGRQMFGAGIDFWGQGTLVTVSS

SEQ ID NO: 38 - protein, 120 aa, Homo sapiens
QVQLVQSGAEVKKPGSSVKVSCKASGGTFWRYAISWVRQAPGQGLEWMGVIIPIWGKANYAQKFQGRVTITADESTSTAYMELSSLRSEDTAVYYCARGRQMFGAGIDFWGQGTLVTVSS

SEQ ID NO: 39 - protein, 120 aa, Homo sapiens
QVQLVQSGAEVKKPGSSVKVSCKASGGTFGSYAISWVRQAPGQGLEWMGGIYPAFGTANYAQKFQGRVTITADESTSTAYMELSSLRSEDTAVYYCARGRQMFGAGIDFWGQGTLVTVSS

SEQ ID NO: 40 - protein, 120 aa, Homo sapiens
QVQLVQSGAEVKKPGSSVKVSCKASGGTFGTYAISWVRQAPGQGLEWMGGIYPRFGTANYAQKFQGRVTITADESTSTAYMELSSLRSEDTAVYYCARGRQMFGAGIDFWGQGTLVTVSS

SEQ ID NO: 41 - protein, 120 aa, Homo sapiens
QVQLVQSGAEVKKPGSSVKVSCKASGGTFSPKAISWVRQAPGQGLEWMGVIIPIFGPANYAQKFQGRVTITADESTSTAYMELSSLRSEDTAVYYCARGRQMFGAGIDFWGQGTLVTVSS

SEQ ID NO: 42 - protein, 112 aa, Homo sapiens
NFMLTQPHSVSESPGKTVTISCTRSSGSIDSNYVQWYQQRPGSAPTTVIYEDNQRPSGVPDRFSGSIDSSSNSASLTISGLKTEDEADYYCQSYDSNNRHVIFGGGTKLTVL

SEQ ID NO: 43 - protein, 26 aa, Homo sapiens
EVQLVQSGGEVKKPGASVKVSCKASG

SEQ ID NO: 44 - protein, 30 aa, Homo sapiens
RVTMTTDTSTNTAYMELRSLTADDTAVYYC

SEQ ID NO: 45 - protein, 22 aa, Homo sapiens
LSVLTQPPSVSVAPGQTARITC

SEQ ID NO: 46 - protein, 15 aa, Homo sapiens
WYQQKPGQAPVLVVY

SEQ ID NO: 47 - protein, 32 aa, Homo sapiens
GIPERFSGSNSGNTATLTISRVEAGDEADYYC

SEQ ID NO: 48 - protein, 120 aa, Homo sapiens
EVQLVQSGGEVKKPGASVKVSCKASGYTLSSHGITWVRQAPGQGLEWMGWISAHSGHASNAQKVEDRVTMTTDTSTNTAYMELRSLTADDTAVYYCARVWRALYHGMDVWGQGTLVTVSS

SEQ ID NO: 49 - protein, 120 aa, Homo sapiens
EVQLVQSGGEVKKPGASVKVSCKASGYTLSSHGITWVRQAPGQGLEWMGWISAHSGHASNAQKVEDRVTMTTDTSTNTAYMELRSLTADDTAVYYCARVHAALYHGMDVWGQGTLVTVSS

SEQ ID NO: 50 - protein, 108 aa, Homo sapiens
LSVLTQPPSVSVAPGQTARITCGGNNIGSKGVHWYQQKPGQAPVLVVYDDSDRPSGIPERFSGSNSGNTATLTISRVEAGDEADYYCQVWDSSSDHWVFGGGTKLTVL

SEQ ID NO: 51 - protein, 120 aa, Homo sapiens
EVQLVQSGAEVKKPGSSVKVSCKASGGTFSRSAISWVRQAPGQGLEWMGVIIPAFGEANYAQKFQGRVTITADESTSTAYMELSSLRSEDTAVYYCARGRQMFGAGIDFWGQGTLVTVSS

SEQ ID NO: 52 - protein, 120 aa, Homo sapiens
EVQLVQSGAEVKKPGSSVKVSCKASGGTFSGYAISWVRQAPGQGLEWMGVIIPAFGTANYAQKFQGRVTITADESTSTAYMELSSLRSEDTAVYYCARGRQMFGAGIDFWGQGTLVTVSS

SEQ ID NO: 53 - protein, 120 aa, Homo sapiens
EVQLVQSGAEVKKPGSSVKVSCKASGGTFWRYAISWVRQAPGQGLEWMGVIIPIWGKANYAQKFQGRVTITADESTSTAYMELSSLRSEDTAVYYCARGRQMFGAGIDFWGQGTLVTVSS

SEQ ID NO: 54 - protein, 120 aa, Homo sapiens
EVQLVQSGAEVKKPGSSVKVSCKASGGTFGSYAISWVRQAPGQGLEWMGGIYPAFGTANYAQKFQGRVTITADESTSTAYMELSSLRSEDTAVYYCARGRQMFGAGIDFWGQGTLVTVSS

SEQ ID NO: 55 - protein, 120 aa, Homo sapiens
EVQLVQSGAEVKKPGSSVKVSCKASGGTFGTYAISWVRQAPGQGLEWMGGIYPRFGTANYAQKFQGRVTITADESTSTAYMELSSLRSEDTAVYYCARGRQMFGAGIDFWGQGTLVTVSS

SEQ ID NO: 56 - protein, 120 aa, Homo sapiens
EVQLVQSGAEVKKPGSSVKVSCKASGGTFSPKAISWVRQAPGQGLEWMGVIIPIFGPANYAQKFQGRVTITADESTSTAYMELSSLRSEDTAVYYCARGRQMFGAGIDFWGQGTLVTVSS

SEQ ID NO: 57 - protein, 13 aa, Homo sapiens
ARVHAALYYGMDV

SEQ ID NO: 58 - protein, 120 aa, Homo sapiens
EVQLVQSGGEVKKPGASVKVSCKASGYTLSSHGITWVRQAPGQGLEWMGWISAHSGHASNAQKVEDRVTMTTDTSTNTAYMELRSLTADDTAVYYCARVHAALYYGMDVWGQGTLVTVSS

SEQ ID NO: 59 - DNA, 360 bp, Homo sapiens
gaggtgcagctggtgcagtctggggctgaggtgaagaagcctgggtcctcggtgaaggtctcctgcaaggcttctggaggcaccttcagcagctatgctatcagctgggtgcgacaggcccctggacaagggcttgagtggatgggagggatcatccctatctttggtacagcaaactacgcacagaagttccagggcagagtcacgattaccgcggacaagtccacgagcacagcctacatggagctgagcagcctgagatctgaggacacggcggtgtactactgcgctagaggcagacagatgttcggtgcaggcatcgatttctggggccagggcaccctggtcaccgtctcctca

SEQ ID NO: 60 - DNA, 360 bp, Homo sapiens
caggtgcagctggtgcagtctggggctgaggtgaagaagcctgggtcctcggtgaaggtctcctgcaaggcttctggaggcaccttcagccgttcggctatcagctgggtgcgacaggcccctggacaagggcttgagtggatgggagttatcatccctgcgtttggtgaggcaaactacgcacagaagttccagggcagagtcacgattaccgcggacgaatccacgagcacagcctacatggagctgagcagcctgagatctgaggacacggcggtgtactactgcgctagaggcagacagatgttcggtgcaggcatcgatttctggggccagggcaccctggtcaccgtctcctca

SEQ ID NO: 61 - DNA, 360 bp, Homo sapiens
caggtgcagctggtgcagtctggggctgaggtgaagaagcctgggtcctcggtgaaggtatcatgcaaggcttctggaggcaccttcagcgggtatgctatctcttgggtgcgacaggcccctggacaagggcttgagtggatgggagttatcatccctgcttttggtacagcaaactacgcacagaagttccagggcagagtcacgattaccgcggacgaatccacgagcacagcctacatggagctgagcagcctgagatctgaggacacggcggtgtactactgcgccagaggcagacagatgttcggtgcaggcatcgatttctggggccagggcaccctggtcaccgtctcctca

SEQ ID NO: 62 - DNA, 360 bp, Homo sapiens
caggtgcagctggtgcagtctggggctgaggtgaagaagcctgggtcctcggtgaaggtctcctgcaaggcttctggaggcaccttctggaggtatgctatcagctgggtgcgacaggcccctggacaagggcttgagtggatgggagttatcatccctatctggggtaaagcaaactacgcacagaagttccagggcagagtcacgattaccgcggacgaatccacgagcacagcctacatggagctgagcagcctgagatctgaggacacggcggtgtactactgcgccagaggcagacagatgttcggtgcaggcatcgatttctggggccagggcaccctggtcaccgtctcctca

SEQ ID NO: 63 - DNA, 360 bp, Homo sapiens
caggtgcagctggtgcagtctggggctgaggtgaagaagcctgggtcctcggtgaaggtctcctgcaaggcttctggaggcaccttcgggagctatgctatctcttgggtgcgacaggcccctggacaagggcttgagtggatgggagggatctatcctgcttttggtacagcaaactacgcacagaagttccagggcagagtcacgattaccgcggacgaatccacgagcacagcctacatggagctgagcagcctgagatctgaggacacggcggtgtactactgcgctagaggcagacagatgttcggtgcaggcatcgatttctggggccagggcaccctggtcaccgtctcctca

SEQ ID NO: 64 - DNA, 360 bp, Homo sapiens
caggtgcagctggtgcagtctggggctgaggtgaagaagcctgggtcctcggtgaaggtctcctgcaaggcttctggaggcaccttcgggacgtatgctatcagctgggtgcgacaggcccctggacaagggcttgagtggatgggagggatctatcctaggtttggtacagcaaactacgcacagaagttccagggcagagtcacgattaccgcggacgaatccacgagcacagcctacatggagctgagcagcctgagatctgaggacacggcggtgtactactgcgctagaggcagacagatgttcggtgcaggcatcgatttctggggccagggcaccctggtcaccgtctcctca

SEQ ID NO: 65 - DNA, 360 bp, Homo sapiens
caggtgcagctggtgcagtctggggctgaggtgaagaagcctgggtcctcggtgaaggtctcctgcaaggcttctggaggcaccttcagcccgaaggctatcagctgggtgcgacaggcccctggacaagggcttgagtggatgggagtgatcatccctatctttggtccggcaaactacgcacagaagttccagggcagagtcacgattaccgcggacgaatccacgagcacagcctacatggagctgagcagcctgagatctgaggacacggcggtgtactactgcgctagaggcagacagatgttcggtgcaggcatcgatttctggggccagggcaccctggtcaccgtctcctca

SEQ ID NO: 66 - DNA, 360 bp, Homo sapiens
gaggttcagctggtgcagtctggaggtgaggtgaagaagcctggggcctcagtgaaggtctcctgcaaggcttctggttacacccttagcagccatggtatcacctgggtgcgacaggcccctggacaagggcttgagtggatgggatggatcagcgctcacagtggtcacgcaagcaatgcacagaaggtcgaggacagagtcaccatgaccacagacacatccacgaacacagcctacatggagctgaggagcctgacagctgacgacacggcggtgtactactgcgccagagtccatgccgccttgtactacggtatggacgtctgggggcaagggaccctggtcaccgtctcctca

SEQ ID NO: 67 - DNA, 360 bp, Homo sapiens
gaggttcagctggtgcagtctggaggtgaggtgaagaagcctggggcctcagtgaaggtctcctgcaaggcttctggttacacccttagcagccatggtatcacctgggtgcgacaggcccctggacaagggcttgagtggatgggatggatcagcgctcacagtggtcacgcaagcaatgcacagaaggtcgaggacagagtcaccatgaccacagacacatccacgaacacagcctacatggagctgaggagcctgacagctgacgacacggcggtgtactactgcgccagagtccatgccgccttgtaccacggtatggacgtctgggggcaagggaccctggtcaccgtctcctca

SEQ ID NO: 68 - DNA, 360 bp, Homo sapiens
gaggttcagctggtgcagtctggaggtgaggtgaagaagcctggggcctcagtgaaggtctcctgcaaggcttctggttacacccttagcagccatggtatcacctgggtgcgacaggcccctggacaagggcttgagtggatgggatggatcagcgctcacagtggtcacgcaagcaatgcacagaaggtcgaggacagagtcaccatgaccacagacacatccacgaacacagcctacatggagctgaggagcctgacagctgacgacacggcggtgtactactgcgccagagtgtggagggccttgtaccacggtatggacgtctgggggcaagggaccctggtcaccgtctcctca

SEQ ID NO: 69 - DNA, 336 bp, Homo sapiens
aattttatgctgactcagccccactctgtgtcggagtctccggggaagacggtaaccatctcctgcacccgcagcagtggcagcattgacagcaactatgtgcagtggtaccagcagcgcccgggcagtgcccccaccactgtgatctatgaggataaccaaagaccctctggggtccctgatcggttctctggctccatcgacagctcctccaactctgcctccctcaccatctctggactgaagactgaggacgaggctgactactactgtcagtcttatgatagcaacaataggcatgtgatattcggcggagggaccaagctgaccgtccta

SEQ ID NO: 70 - DNA, 324 bp, Homo sapiens
ttgtctgtgctgactcagccaccctcagtgtcagtggccccaggacagacggccaggattacctgtgggggaaacaacattggaagtaaaggtgtgcactggtaccagcagaagccaggccaggcccctgtgctggtcgtctatgatgatagcgaccggccctcagggatccctgagcgattctctggctccaactctgggaacacggccaccctgaccatcagcagggtcgaagccggggatgaggccgactattactgtcaggtgtgggacagtagtagtgatcattgggtgttcggcggagggaccaagctgaccgtccta

SEQ ID NO: 71 - protein, 120 aa, Homo sapiens
QVQLVQSGAEVKKPGSSVKVSCKASGGTFSSYAISWVRQAPGQGLEWMGGIIPIFGTANYAQKFQGRVTITADKSTSTAYMELSSLRSEDTAVYYCARGRQMFGAGIDFWGQGTLVTVSS

SEQ ID NO: 72 - protein, 120 aa, Homo sapiens; identical to SEQ ID NO: 58

SEQ ID NO: 73 - protein, 451 aa, Homo sapiens
EVQLVESGGGLVQPGGSLRLSCAASGFTFSRYWMSWVRQAPGKGLEWVANIKQDGSEKYYVDSVKGRFTISRDNAKNSLYLQMNSLRAEDTAVYYCAREGGWFGELAFDYWGQGTLVTVSSASTKGPSVFPLAPSSKSTSGGTAALGCLVKDYFPEPVTVSWNSGALTSGVHTFPAVLQSSGLYSLSSVVTVPSSSLGTQTYICNVNHKPSNTKVDKRVEPKSCDKTHTCPPCPAPEFEGGPSVFLFPPKPKDTLMISRTPEVTCVVVDVSHEDPEVKFNWYVDGVEVHNAKTKPREEQYNSTYRVVSVLTVLHQDWLNGKEYKCKVSNKALPASIEKTISKAKGQPREPQVYTLPPSREEMTKNQVSLTCLVKGFYPSDIAVEWESNGQPENNYKTTPPVLDSDGSFFLYSKLTVDKSRWQQGNVFSCSVMHEALHNHYTQKSLSLSPGK

SEQ ID NO: 74 - protein, 215 aa, Homo sapiens
EIVLTQSPGTLSLSPGERATLSCRASQRVSSSYLAWYQQKPGQAPRLLIYDASSRATGIPDRFSGSGSGTDFTLTISRLEPEDFAVYYCQQYGSLPWTFGQGTKVEIKRTVAAPSVFIFPPSDEQLKSGTASVVCLLNNFYPREAKVQWKVDNALQSGNSQESVTEQDSKDSTYSLSSTLTLSKADYEKHKVYACEVTHQGLSSPVTKSFNRGEC

SEQ ID NO: 75 - protein, 11 aa, Homo sapiens
QSYDSNLRHVI

SEQ ID NO: 76 - protein, 11 aa, Homo sapiens
QSYDSNIRHVI

SEQ ID NO: 77 - protein, 34 aa, Homo sapiens
GVPDRFSGSIDSSSNWASLTISGLKTEDEADYYC

SEQ ID NO: 78 - protein, 34 aa, Homo sapiens
GVPDRFSGSIDSSSNVASLTISGLKTEDEADYYC